European Patent Application EP 4 501 338 A1, published February 5, 2025. Title: A medical compound which includes miR-140 and a method for manufacturing thereof. Applicant: Regenesis Science, Inc. Application JP. The sequence listing filed with the application follows.

SEQUENCE LISTING (2 sequences)

SEQ ID NO: 1 - DNA, 20 bp, synthetic construct
  misc_feature 1..20: note = Primer
  source 1..20: mol_type = other DNA
gactcagggcatgaaacagg

SEQ ID NO: 2 - DNA, 19 bp, synthetic construct
  misc_feature 1..19: note = Primer
  source 1..19: mol_type = other DNA
actgaggggcctgaaatga